European Patent Specification EP 2 752 200 B1, published November 1, 2023. Title: Antigen-binding molecules inducing immune responses against target antigens. Applicant: CHUGAI SEIYAKU KABUSHIKI KAISHA. The sequence listing filed with the application follows.

SEQUENCE LISTING (138 sequences)

SEQ ID NO: 1 - protein, 468 aa, Homo sapiens
MLAVGCALLAALLAAPGAALAPRRCPAQEVARGVLTSLPGDSVTLTCPGVEPEDNATVHWVLRKPAAGSHPSRWAGMGRRLLLRSVQLHDSGNYSCYRAGRPAGTVHLLVDVPPEEPQLSCFRKSPLSNVVCEWGPRSTPSLTTKAVLLVRKFQNSPAEDFQEPCQYSQESQKFSCQLAVPEGDSSFYIVSMCVASSVGSKFSKTQTFQGCGILQPDPPANITVTAVARNPRWLSVTWQDPHSWNSSFYRLRFELRYRAERSKTFTTWMVKDLQHHCVIHDAWSGLRHVVQLRAQEEFGQGEWSEWSPEAMGTPWTESRSPPAENEVSTPMQALTTNKDDDNILFRDSANATSLPVQDSSSVPLPTFLVAGGSLAFGTLLCIAIVLRFKKTWKLRALKEGKTSMHPPYSLGQLVPERPRPTPVLVPLISPPVSPSSLGSDNTSSHNRPDARDPRSPYDISNTDYFFPR

SEQ ID NO: 2 - DNA, 1407 bp, Homo sapiens
atgctggccgtcggctgcgcgctgctggctgccctgctggccgcgccgggagcggcgctggccccaaggcgctgccctgcgcaggaggtggcgagaggcgtgctgaccagtctgccaggagacagcgtgactctgacctgcccgggggtagagccggaagacaatgccactgttcactgggtgctcaggaagccggctgcaggctcccaccccagcagatgggctggcatgggaaggaggctgctgctgaggtcggtgcagctccacgactctggaaactattcatgctaccgggccggccgcccagctgggactgtgcacttgctggtggatgttccccccgaggagccccagctctcctgcttccggaagagccccctcagcaatgttgtttgtgagtggggtcctcggagcaccccatccctgacgacaaaggctgtgctcttggtgaggaagtttcagaacagtccggccgaagacttccaggagccgtgccagtattcccaggagtcccagaagttctcctgccagttagcagtcccggagggagacagctctttctacatagtgtccatgtgcgtcgccagtagtgtcgggagcaagttcagcaaaactcaaacctttcagggttgtggaatcttgcagcctgatccgcctgccaacatcacagtcactgccgtggccagaaacccccgctggctcagtgtcacctggcaagacccccactcctggaactcatctttctacagactacggtttgagctcagatatcgggctgaacggtcaaagacattcacaacatggatggtcaaggacctccagcatcactgtgtcatccacgacgcctggagcggcctgaggcacgtggtgcagcttcgtgcccaggaggagttcgggcaaggcgagtggagcgagtggagcccggaggccatgggcacgccttggacagaatccaggagtcctccagctgagaacgaggtgtccacccccatgcaggcacttactactaataaagacgatgataatattctcttcagagattctgcaaatgcgacaagcctcccagtgcaagattcttcttcagtaccactgcccacattcctggttgctggagggagcctggccttcggaacgctcctctgcattgccattgttctgaggttcaagaagacgtggaagctgcgggctctgaaggaaggcaagacaagcatgcatccgccgtactctttggggcagctggtcccggagaggcctcgacccaccccagtgcttgttcctctcatctccccaccggtgtcccccagcagcctggggtctgacaatacctcgagccacaaccgaccagatgccagggacccacggagcccttatgacatcagcaatacagactacttcttccccagatag

SEQ ID NO: 3 - protein, 19 aa, Artificial sequence
  An artificially synthesized peptide sequence
MGWSCIILFLVATATGVHS

SEQ ID NO: 4 - protein, 214 aa, Artificial sequence
  An artificially synthesized peptide sequence
ETTLTQSPAFMSATPGDKVNISCKASQDIDDDMNWYQQKPGEAAIFIIQEATTLVPGISPRFSGSGYGTDFTLTINNIESEDAAYYFCLQHDNFPYTFGQGTKLEIKRTVAAPSVFIFPPSDEQLKSGTASVVCLLNNFYPREAKVQWKVDNALQSGNSQESVTEQDSKDSTYSLSSTLTLSKADYEKHKVYACEVTHQGLSSPVTKSFNRGEC

SEQ ID NO: 5 - protein, 107 aa, Artificial sequence
  An artificially synthesized peptide sequence
DIQMTQSPSSLSASVGDRVTITCRASQSISSYLNWYQQKPGKAPKLLIYAASSLQSGVPSRFSGSGSGTDFTLTISSLQPEDFATYYCQQSYSTPFTFGPGTKVDIK

SEQ ID NO: 6 - protein, 112 aa, Artificial sequence
  An artificially synthesized peptide sequence
DIVMTQSPLSLPVTPGEPASISCRSSQSLLHSNGDNYLDWYLQKPGQSPQLLIYLGSNRASGVPDRFSGSGSGTDFTLKISRVEAEDVGVYYCMQVLRNPLTFGGGTKVEIQ

SEQ ID NO: 7 - protein, 107 aa, Artificial sequence
  An artificially synthesized peptide sequence
EIVMTQSPATLSLSPGERATLSCRASQSVSSYLAWYQQKPGQAPRLLIYDASNRATGIPARFSGSGSGTDFTLTISSLEPEDFAVYYCQQRSNWPPTFGQGTKVEIK

SEQ ID NO: 8 - protein, 112 aa, Artificial sequence
  An artificially synthesized peptide sequence
DIVMTQSPESLVLSLGGTATINCRSSQSVLYSSNNKNYLTWYQQKPGQPPTLLFSWASIRDSGVPDRFSASGSGTEFTLTISDLQAEDAAVYYCQQYYRAPSFGQGTKLQIK

SEQ ID NO: 9 - protein, 449 aa, Artificial sequence
  An artificially synthesized peptide sequence
QVQLVQSGAEVKKPGASVKVSCKASGYTFTSYYMHWVRQAPGQGLEWMGIINPSGGSTSYAQKFQGRVTMTRDTSTSTVYMELSSLRSEDTAVYYCARDDPGGGEYYFDYWGQGTLVTVSSASTKGPSVFPLAPSSKSTSGGTAALGCLVKDYFPEPVTVSWNSGALTSGVHTFPAVLQSSGLYSLSSVVTVPSSSLGTQTYICNVNHKPSNTKVDKKVEPKSCDKTHTCPPCPAPELLGGPSVFLFPPKPKDTLMISRTPEVTCVVVDVSHEDPEVKFNWYVDGVEVHNAKTKPREEQYNSTYRVVSVLTVLHQDWLNGKEYKCKVSNKALPAPIEKTISKAKGQPREPQVYTLPPSRDELTKNQVSLTCLVKGFYPSDIAVEWESNGQPENNYKTTPPVLDSDGSFFLYSKLTVDKSRWQQGNVFSCSVMHEALHNHYTQKSLSLSP

SEQ ID NO: 10 - protein, 126 aa, Artificial sequence
  An artificially synthesized peptide sequence
EVQLVESGGGLVQPGGSLRLSCAASGFTFSSYEMNWVRQAPGKGLEWVSYISSSGSTIYYADSVKGRFTISRDNAKNSLYLQMNSLRAEDTAVYYCARDAPYYYDSSGYTDAFDIWGQGTMVTVSS

SEQ ID NO: 11 - protein, 330 aa, Homo sapiens [sequence omitted]

SEQ ID NO: 12 - protein, 326 aa, Homo sapiens
ASTKGPSVFPLAPCSRSTSESTAALGCLVKDYFPEPVTVSWNSGALTSGVHTFPAVLQSSGLYSLSSVVTVPSSNFGTQTYTCNVDHKPSNTKVDKTVERKCCVECPPCPAPPVAGPSVFLFPPKPKDTLMISRTPEVTCVVVDVSHEDPEVQFNWYVDGVEVHNAKTKPREEQFNSTFRVVSVLTVVHQDWLNGKEYKCKVSNKGLPAPIEKTISKTKGQPREPQVYTLPPSREEMTKNQVSLTCLVKGFYPSDIAVEWESNGQPENNYKTTPPMLDSDGSFFLYSKLTVDKSRWQQGNVFSCSVMHEALHNHYTQKSLSLSPGK

SEQ ID NO: 13 - protein, 377 aa, Homo sapiens
ASTKGPSVFPLAPCSRSTSGGTAALGCLVKDYFPEPVTVSWNSGALTSGVHTFPAVLQSSGLYSLSSVVTVPSSSLGTQTYTCNVNHKPSNTKVDKRVELKTPLGDTTHTCPRCPEPKSCDTPPPCPRCPEPKSCDTPPPCPRCPEPKSCDTPPPCPRCPAPELLGGPSVFLFPPKPKDTLMISRTPEVTCVVVDVSHEDPEVQFKWYVDGVEVHNAKTKPREEQYNSTFRVVSVLTVLHQDWLNGKEYKCKVSNKALPAPIEKTISKTKGQPREPQVYTLPPSREEMTKNQVSLTCLVKGFYPSDIAVEWESSGQPENNYNTTPPMLDSDGSFFLYSKLTVDKSRWQQGNIFSCSVMHEALHNRFTQKSLSLSPGK

SEQ ID NO: 14 - protein, 327 aa, Homo sapiens
ASTKGPSVFPLAPCSRSTSESTAALGCLVKDYFPEPVTVSWNSGALTSGVHTFPAVLQSSGLYSLSSVVTVPSSSLGTKTYTCNVDHKPSNTKVDKRVESKYGPPCPSCPAPEFLGGPSVFLFPPKPKDTLMISRTPEVTCVVVDVSQEDPEVQFNWYVDGVEVHNAKTKPREEQFNSTYRVVSVLTVLHQDWLNGKEYKCKVSNKGLPSSIEKTISKAKGQPREPQVYTLPPSQEEMTKNQVSLTCLVKGFYPSDIAVEWESNGQPENNYKTTPPVLDSDGSFFLYSRLTVDKSRWQEGNVFSCSVMHEALHNHYTQKSLSLSLGK

SEQ ID NO: 15 - protein, 365 aa, Homo sapiens
MGVPRPQPWALGLLLFLLPGSLGAESHLSLLYHLTAVSSPAPGTPAFWVSGWLGPQQYLSYNSLRGEAEPCGAWVWENQVSWYWEKETTDLRIKEKLFLEAFKALGGKGPYTLQGLLGCELGPDNTSVPTAKFALNGEEFMNFDLKQGTWGGDWPEALAISQRWQQQDKAANKELTFLLFSCPHRLREHLERGRGNLEWKEPPSMRLKARPSSPGFSVLTCSAFSFYPPELQLRFLRNGLAAGTGQGDFGPNSDGSFHASSSLTVKSGDEHHYCCIVQHAGLAQPLRVELESPAKSSVLVVGIVIGVLLLTAAAVGGALLWRRMRSGLPAPWISLRGDDTGVLLPTPGEAQDADLKDVNVIPATA

SEQ ID NO: 16 - protein, 119 aa, Homo sapiens
MSRSVALAVLALLSLSGLEAIQRTPKIQVYSRHPAENGKSNFLNCYVSGFHPSDIEVDLLKNGERIEKVEHSDLSFSKDWSFYLLYYTEFTPTEKDEYACRVNHVTLSQPKIVKWDRDM

SEQ ID NO: 17 - protein, 447 aa, Artificial sequence
  An artificially synthesized peptide sequence
QVQLQESGPGLVKPSETLSLTCAVSGHSISHDHAWSWVRQPPGEGLEWIGFISYSGITNYNPSLQGRVTISRDNSKNTLYLQMNSLRAEDTAVYYCARSLARTTAMDYWGEGTLVTVSSASTKGPSVFPLAPSSKSTSGGTAALGCLVKDYFPEPVTVSWNSGALTSGVHTFPAVLQSSGLYSLSSVVTVPSSSLGTQTYICNVNHKPSNTKVDKKVEPKSCDKTHTCPPCPAPELLGGPSVFLFPPKPKDTLMISRTPEVTCVVVDVSHEDPEVKFNWYVDGVEVHNAKTKPREEQYNSTYRVVSVLTVLHQDWLNGKEYKCKVSNKALPAPIEKTISKAKGQPREPQVYTLPPSRDELTKNQVSLTCLVKGFYPSDIAVEWESNGQPENNYKTTPPVLDSDGSFFLYSKLTVDKSRWQQGNVFSCSVMHEALHNHYTQKSLSLSP

SEQ ID NO: 18 - protein, 214 aa, Artificial sequence [sequence omitted]

SEQ ID NO: 19 - DNA, 1125 bp, Homo sapiens
atgtggttcttgacaactctgctcctttgggttccagttgatgggcaagtggacaccacaaaggcagtgatcactttgcagcctccatgggtcagcgtgttccaagaggaaaccgtaaccttgcactgtgaggtgctccatctgcctgggagcagctctacacagtggtttctcaatggcacagccactcagacctcgacccccagctacagaatcacctctgccagtgtcaatgacagtggtgaatacaggtgccagagaggtctctcagggcgaagtgaccccatacagctggaaatccacagaggctggctactactgcaggtctccagcagagtcttcacggaaggagaacctctggccttgaggtgtcatgcgtggaaggataagctggtgtacaatgtgctttactatcgaaatggcaaagcctttaagtttttccactggaattctaacctcaccattctgaaaaccaacataagtcacaatggcacctaccattgctcaggcatgggaaagcatcgctacacatcagcaggaatatctgtcactgtgaaagagctatttccagctccagtgctgaatgcatctgtgacatccccactcctggaggggaatctggtcaccctgagctgtgaaacaaagttgctcttgcagaggcctggtttgcagctttacttctccttctacatgggcagcaagaccctgcgaggcaggaacacatcctctgaataccaaatactaactgctagaagagaagactctgggttatactggtgcgaggctgccacagaggatggaaatgtccttaagcgcagccctgagttggagcttcaagtgcttggcctccagttaccaactcctgtctggtttcatgtccttttctatctggcagtgggaataatgtttttagtgaacactgttctctgggtgacaatacgtaaagaactgaaaagaaagaaaaagtgggatttagaaatctctttggattctggtcatgagaagaaggtaatttccagccttcaagaagacagacatttagaagaagagctgaaatgtcaggaacaaaaagaagaacagctgcaggaaggggtgcaccggaaggagccccagggggccacgtag

SEQ ID NO: 20 - protein, 374 aa, Homo sapiens
MWFLTTLLLWVPVDGQVDTTKAVITLQPPWVSVFQEETVTLHCEVLHLPGSSSTQWFLNGTATQTSTPSYRITSASVNDSGEYRCQRGLSGRSDPIQLEIHRGWLLLQVSSRVFTEGEPLALRCHAWKDKLVYNVLYYRNGKAFKFFHWNSNLTILKTNISHNGTYHCSGMGKHRYTSAGISVTVKELFPAPVLNASVTSPLLEGNLVTLSCETKLLLQRPGLQLYFSFYMGSKTLRGRNTSSEYQILTARREDSGLYWCEAATEDGNVLKRSPELELQVLGLQLPTPVWFHVLFYLAVGIMFLVNTVLWVTIRKELKRKKKWDLEISLDSGHEKKVISSLQEDRHLEEELKCQEQKEEQLQEGVHRKEPQGAT

SEQ ID NO: 21 - DNA, 951 bp, Homo sapiens
atgactatggagacccaaatgtctcagaatgtatgtcccagaaacctgtggctgcttcaaccattgacagttttgctgctgctggcttctgcagacagtcaagctgctcccccaaaggctgtgctgaaacttgagcccccgtggatcaacgtgctccaggaggactctgtgactctgacatgccagggggctcgcagccctgagagcgactccattcagtggttccacaatgggaatctcattcccacccacacgcagcccagctacaggttcaaggccaacaacaatgacagcggggagtacacgtgccagactggccagaccagcctcagcgaccctgtgcatctgactgtgctttccgaatggctggtgctccagacccctcacctggagttccaggagggagaaaccatcatgctgaggtgccacagctggaaggacaagcctctggtcaaggtcacattcttccagaatggaaaatcccagaaattctcccatttggatcccaccttctccatcccacaagcaaaccacagtcacagtggtgattaccactgcacaggaaacataggctacacgctgttctcatccaagcctgtgaccatcactgtccaagtgcccagcatgggcagctcttcaccaatgggggtcattgtggctgtggtcattgcgactgctgtagcagccattgttgctgctgtagtggccttgatctactgcaggaaaaagcggatttcagccaattccactgatcctgtgaaggctgcccaatttgagccacctggacgtcaaatgattgccatcagaaagagacaacttgaagaaaccaacaatgactatgaaacagctgacggcggctacatgactctgaaccccagggcacctactgacgatgataaaaacatctacctgactcttcctcccaacgaccatgtcaacagtaataactaa

SEQ ID NO: 22 - protein, 316 aa, Homo sapiens
MTMETQMSQNVCPRNLWLLQPLTVLLLLASADSQAAPPKAVLKLEPPWINVLQEDSVTLTCQGARSPESDSIQWFHNGNLIPTHTQPSYRFKANNNDSGEYTCQTGQTSLSDPVHLTVLSEWLVLQTPHLEFQEGETIMLRCHSWKDKPLVKVTFFQNGKSQKFSHLDPTFSIPQANHSHSGDYHCTGNIGYTLFSSKPVTITVQVPSMGSSSPMGVIVAVVIATAVAAIVAAVVALIYCRKKRISANSTDPVKAAQFEPPGRQMIAIRKRQLEETNNDYETADGGYMTLNPRAPTDDDKNIYLTLPPNDHVNSNN

SEQ ID NO: 23 - DNA, 876 bp, Homo sapiens
atgggaatcctgtcattcttacctgtccttgccactgagagtgactgggctgactgcaagtccccccagccttggggtcatatgcttctgtggacagctgtgctattcctggctcctgttgctgggacacctgcagctcccccaaaggctgtgctgaaactcgagccccagtggatcaacgtgctccaggaggactctgtgactctgacatgccgggggactcacagccctgagagcgactccattcagtggttccacaatgggaatctcattcccacccacacgcagcccagctacaggttcaaggccaacaacaatgacagcggggagtacacgtgccagactggccagaccagcctcagcgaccctgtgcatctgactgtgctttctgagtggctggtgctccagacccctcacctggagttccaggagggagaaaccatcgtgctgaggtgccacagctggaaggacaagcctctggtcaaggtcacattcttccagaatggaaaatccaagaaattttcccgttcggatcccaacttctccatcccacaagcaaaccacagtcacagtggtgattaccactgcacaggaaacataggctacacgctgtactcatccaagcctgtgaccatcactgtccaagctcccagctcttcaccgatggggatcattgtggctgtggtcactgggattgctgtagcggccattgttgctgctgtagtggccttgatctactgcaggaaaaagcggatttcagccaatcccactaatcctgatgaggctgacaaagttggggctgagaacacaatcacctattcacttctcatgcacccggatgctctggaagagcctgatgaccagaaccgtatttag

SEQ ID NO: 24 - protein, 291 aa, Homo sapiens
MGILSFLPVLATESDWADCKSPQPWGHMLLWTAVLFLAPVAGTPAAPPKAVLKLEPQWINVLQEDSVTLTCRGTHSPESDSIQWFHNGNLIPTHTQPSYRFKANNNDSGEYTCQTGQTSLSDPVHLTVLSEWLVLQTPHLEFQEGETIVLRCHSWKDKPLVKVTFFQNGKSKKFSRSDPNFSIPQANHSHSGDYHCTGNIGYTLYSSKPVTITVQAPSSSPMGIIVAVVTGIAVAAIVAAVVALIYCRKKRISANPTNPDEADKVGAENTITYSLLMHPDALEEPDDQNRI

SEQ ID NO: 25 - DNA, 765 bp, Homo sapiens
atgtggcagctgctcctcccaactgctctgctacttctagtttcagctggcatgcggactgaagatctcccaaaggctgtggtgttcctggagcctcaatggtacagggtgctcgagaaggacagtgtgactctgaagtgccagggagcctactcccctgaggacaattccacacagtggtttcacaatgagagcctcatctcaagccaggcctcgagctacttcattgacgctgccacagttgacgacagtggagagtacaggtgccagacaaacctctccaccctcagtgacccggtgcagctagaagtccatatcggctggctgttgctccaggcccctcggtgggtgttcaaggaggaagaccctattcacctgaggtgtcacagctggaagaacactgctctgcataaggtcacatatttacagaatggcaaaggcaggaagtattttcatcataattctgacttctacattccaaaagccacactcaaagacagcggctcctacttctgcagggggcttgttgggagtaaaaatgtgtcttcagagactgtgaacatcaccatcactcaaggtttgtcagtgtcaaccatctcatcattctttccacctgggtaccaagtctctttctgcttggtgatggtactcctttttgcagtggacacaggactatatttctctgtgaagacaaacattcgaagctcaacaagagactggaaggaccataaatttaaatggagaaaggaccctcaagacaaatga

SEQ ID NO: 26 - protein, 254 aa, Homo sapiens [sequence omitted]

SEQ ID NO: 27 - DNA, 702 bp, Homo sapiens
atgtggcagctgctcctcccaactgctctgctacttctagtttcagctggcatgcggactgaagatctcccaaaggctgtggtgttcctggagcctcaatggtacagcgtgcttgagaaggacagtgtgactctgaagtgccagggagcctactcccctgaggacaattccacacagtggtttcacaatgagagcctcatctcaagccaggcctcgagctacttcattgacgctgccacagtcaacgacagtggagagtacaggtgccagacaaacctctccaccctcagtgacccggtgcagctagaagtccatatcggctggctgttgctccaggcccctcggtgggtgttcaaggaggaagaccctattcacctgaggtgtcacagctggaagaacactgctctgcataaggtcacatatttacagaatggcaaagacaggaagtattttcatcataattctgacttccacattccaaaagccacactcaaagatagcggctcctacttctgcagggggcttgttgggagtaaaaatgtgtcttcagagactgtgaacatcaccatcactcaaggtttggcagtgtcaaccatctcatcattctctccacctgggtaccaagtctctttctgcttggtgatggtactcctttttgcagtggacacaggactatatttctctgtgaagacaaacatttga

SEQ ID NO: 28 - protein, 233 aa, Homo sapiens
MWQLLLPTALLLLVSAGMRTEDLPKAVVFLEPQWYSVLEKDSVTLKCQGAYSPEDNSTQWFHNESLISSQASSYFIDAATVNDSGEYRCQTNLSTLSDPVQLEVHIGWLLLQAPRWVFKEEDPIHLRCHSWKNTALHKVTYLQNGKDRKYFHHNSDFHIPKATLKDSGSYFCRGLVGSKNVSSETVNITITQGLAVSTISSFSPPGYQVSFCLVMVLLFAVDTGLYFSVKTNI

SEQ ID NO: 29 - protein, 4 aa, Artificial sequence
  An artificially synthesized peptide sequence
GGGS

SEQ ID NO: 30 - protein, 4 aa, Artificial sequence
  An artificially synthesized peptide sequence
SGGG

SEQ ID NO: 31 - protein, 5 aa, Artificial sequence
  An artificially synthesized peptide sequence
GGGGS

SEQ ID NO: 32 - protein, 5 aa, Artificial sequence
  An artificially synthesized peptide sequence
SGGGG

SEQ ID NO: 33 - protein, 6 aa, Artificial sequence
  An artificially synthesized peptide sequence
GGGGGS

SEQ ID NO: 34 - protein, 6 aa, Artificial sequence
  An artificially synthesized peptide sequence
SGGGGG

SEQ ID NO: 35 - protein, 7 aa, Artificial sequence
  An artificially synthesized peptide sequence
GGGGGGS

SEQ ID NO: 36 - protein, 7 aa, Artificial sequence
  An artificially synthesized peptide sequence
SGGGGGG

SEQ ID NO: 37 - protein, 107 aa, Artificial sequence [sequence omitted]

SEQ ID NO: 38 - protein, 447 aa, Artificial sequence
  An artificially synthesized peptide sequence
QVQLQESGPGLVKPSETLSLTCAVSGYSISDDQAWSWVRQPPGEGLEWIGYISYSGITNYNPSLKGRVTISRDTSKNQFSLKLSSVTAADTAAYYCARSLARTTAMDYWGEGTLVTVSSASTKGPSVFPLAPSSKSTSGGTAALGCLVKDYFPEPVTVSWNSGALTSGVHTFPAVLQSSGLYSLSSVVTVPSSSLGTQTYICNVNHKPSNTKVDKKVEPKSCDKTHTCPPCPAPELLGGPSVFLFPPKPKDTLMISRTPEVTCVVVDVSHEDPEVKFNWYVDGVEVHNAKTKPREEQYNSTYRVVSVLTVLHQDWLNGKEYKCKVSNKALPAPIEKTISKAKGQPREPQVYTLPPSRDELTKNQVSLTCLVKGFYPSDIAVEWESNGQPENNYKTTPPVLDSDGSFFLYSKLTVDKSRWQQGNVFSCSVMHEALHNHYTQKSLSLSP

SEQ ID NO: 39 - protein, 214 aa, Artificial sequence
  An artificially synthesized peptide sequence
DIQMTQSPSSLSASVGDSVTITCQASQDISSYLNWYQQKPGKAPELLIYYGSELHSGVPSRFSGSGSGTDFTFTISSLEAEDAATYYCQQGNSLPYTFGQGTKVEIERTVAAPSVFIFPPSDEQLKSGTASVVCLLNNFYPREAKVQWKVDNALQSGNSQESVTEQDSKDSTYSLSSTLTLSKADYEKHKVYACEVTHQGLSSPVTKSFNRGEC

SEQ ID NO: 40 - protein, 214 aa, Artificial sequence
  An artificially synthesized peptide sequence
DIQMTQSPSSLSASVGDSVTITCQASTDISSHLNWYQQKPGKAPELLIYYGSHLLSGVPSRFSGSGSGTDFTFTISSLEAEDAATYYCGQGNRLPYTFGQGTKVEIERTVAAPSVFIFPPSDEQLKSGTASVVCLLNNFYPREAKVQWKVDNALQSGNSQESVTEQDSKDSTYSLSSTLTLSKADYEKHKVYACEVTHQGLSSPVTKSFNRGEC

SEQ ID NO: 41 - protein, 447 aa, Artificial sequence
  An artificially synthesized peptide sequence
QVQLQESGPGLVKPSETLSLTCAVSGYSISDDQAWSWVRQPPGEGLEWIGYISYSGITNYNPSLKGRVTISRDTSKNQFSLKLSSVTAADTAAYYCARSLARTTAMDYWGEGTLVTVSSASTKGPSVFPLAPSSKSTSGGTAALGCLVKDYFPEPVTVSWNSGALTSGVHTFPAVLQSSGLYSLSSVVTVPSSSLGTQTYICNVNHKPSNTKVDKKVEPKSCDKTHTCPPCPAPELLGGPSVFLFPPKPKDTLMISRTAEVTCVVVDVSHEDPEVKFNWYVDGVEVHNAKTKPREEQYNSTYRVVSVLTPLHQDWLNGKEYKCKVSNKALPAPIEKTISKAKGQPREPQVYTLPPSRDELTKNQVSLTCLVKGFYPSDIAVEWESNGQPENNYKTTPPVLDSDGSFFLYSKLTVDKSRWQQGNVFSCSVLHEALHYHYTQKSLSLSP

SEQ ID NO: 42 - protein, 447 aa, Artificial sequence
  An artificially synthesized peptide sequence
QVQLQESGPGLVKPSETLSLTCAVSGHSISHDHAWSWVRQPPGEGLEWIGFISYSGITNYNPSLQGRVTISRDNSKNTLYLQMNSLRAEDTAVYYCARSLARTTAMDYWGEGTLVTVSSASTKGPSVFPLAPSSKSTSGGTAALGCLVKDYFPEPVTVSWNSGALTSGVHTFPAVLQSSGLYSLSSVVTVPSSSLGTQTYICNVNHKPSNTKVDKKVEPKSCDKTHTCPPCPAPELLGGPSVFLFPPKPKDTLMISRTAEVTCVVVDVSHEDPEVKFNWYVDGVEVHNAKTKPREEQYNSTYRVVSVLTPLHQDWLNGKEYKCKVSNKALPAPIEKTISKAKGQPREPQVYTLPPSRDELTKNQVSLTCLVKGFYPSDIAVEWESNGQPENNYKTTPPVLDSDGSFFLYSKLTVDKSRWQQGNVFSCSVLHEALHYHYTQKSLSLSP

SEQ ID NO: 43 - protein, 107 aa, Artificial sequence
  An artificially synthesized peptide sequence
ETTLTQSPAFMSATPGDKVNISCKASQDIDDDMNWYQQKPGEAAIFIIQEATTLVPGISPRFSGSGYGTDFTLTINNIESEDAAYYFCLQHDNFPYTFGQGTKLEIK

SEQ ID NO: 44 - protein, 107 aa, Artificial sequence [sequence omitted]

SEQ ID NO: 45 - protein, 445 aa, Artificial sequence
  An artificially synthesized peptide sequence
QVQLVQSGAEVKKPGASVKVSCKASGYTFTGYIMNWVRQAPGQGLEWMGLINPYNGGTDYNPQFQDRVTITADKSTSTAYMELSSLRSEDTAVYYCARDGYDDGPYTLETWGQGTLVTVSSASTKGPSVFPLAPSSKSTSGGTAALGCLVKDYFPEPVTVSWNSGALTSGVHTFPAVLQSSGLYSLSSVVTVPSSNFGTQTYTCNVDHKPSNTKVDKTVERKSCVECPPCPAPPVAGPSVFLFPPKPKDTLMISRTPEVTCVVVDVSQEDPEVQFNWYVDGVEVHNAKTKPREEQFNSTFRVVSVLTVVHQDWLNGKEYKCKVSNKGLPAPIEKTISKTKGQPREPQVYTLPPSQEEMTKNQVSLTCLVKGFYPSDIAVEWESNGQPENNYKTTPPMLDSDGSFFLYSKLTVDKSRWQEGNVFSCSVMHEALHNHYTQKSLSLSP

SEQ ID NO: 46 - protein, 128 aa, Artificial sequence
  An artificially synthesized peptide sequence
QVQLVQSGAEVKKPGASVKVSCKASGYTFTSYYMHWVRQAPGQGLEWMGIINPSGGSTSYAQKFQGRVTMTRDTSTSTVYMELSSLRSEDTAVYYCARDGTLYDFWSGYYSYDAFDIWGQGTMVTVSS

SEQ ID NO: 47 - protein, 122 aa, Artificial sequence
  An artificially synthesized peptide sequence
QMQLVQSGAEVKKPGSSVKVSCKASGGTFSSYAISWVRQAPGQGLEWMGGIIPIFGTANYAQKFQGRVTITADESTSTAYMELSSLRSEDTAVYYCARDLDTGPYYYGMDVWGQGTMVTVSS

SEQ ID NO: 48 - protein, 124 aa, Artificial sequence
  An artificially synthesized peptide sequence
QVQLVQSGAEVKKPGSSVKVSCKASGGTFSSYAISWVRQAPGQGLEWMGGIIPIFGTANYAQKFQGRVTITADESTSTAYMELSSLRSEDTAVYYCARDSPVPGVYYYYGMDVWGQGTMVTVSS

SEQ ID NO: 49 - protein, 119 aa, Artificial sequence
  An artificially synthesized peptide sequence
QVQLVQSGAEVKKPGESLKISCKGSGYSFTSYWIGWVRQMPGKGLEWMGIIYPGDSDTRYSPSFQGQVTISADKSISTAYLQWSSLKASDTAMYYCARHRAGDLGGDYWGQGTLVTVSS

SEQ ID NO: 50 - protein, 214 aa, Artificial sequence; identical to SEQ ID NO: 4
  An artificially synthesized peptide sequence

SEQ ID NO: 51 - protein, 214 aa, Artificial sequence; identical to SEQ ID NO: 4
  An artificially synthesized peptide sequence

SEQ ID NO: 52 - protein, 214 aa, Artificial sequence
  An artificially synthesized peptide sequence
ETTLTQSPAFMSATPGDKVNISCKASQDIEDDMNWYQQKPGEAAIFIIQEATTLVPGISPRFSGSGYGTDFTLTINNIESEDAAYYFCLQHDNFPLTFGQGTKVEIKRTVAAPSVFIFPPSDEQLKSGTASVVCLLNNFYPREAKVQWKVDNALQSGNSQESVTEQDSKDSTYSLSSTLTLSKADYEKHKVYACEVTHQGLSSPVTKSFNRGEC

SEQ ID NO: 53 - protein, 214 aa, Artificial sequence
  An artificially synthesized peptide sequence
ETTLTQSPAFMSATPGDKVTISCKASQDIDDDMNWYQQKPGEAAIFIIQEATTLVPGISPRFSGSGYGTDFTLTINNIESEDAAYYFCLQHDNFPYTFGQGTKLEIKRTVAAPSVFIFPPSDEQLKSGTASVVCLLNNFYPREAKVQWKVDNALQSGNSQESVTEQDSKDSTYSLSSTLTLSKADYEKHKVYACEVTHQGLSSPVTKSFNRGEC

SEQ ID NO: 54 - protein, 107 aa, Artificial sequence
  An artificially synthesized peptide sequence
DIQMTQSPSSLSASVGDRVTITCKASQDIDDDMNWYQQKPGKAPKLLIYEATTLVPGVPSRFSGSGSGTDFTLTISSLQPEDFATYYCLQHDNFPYTFGQGTKVEIK

SEQ ID NO: 55 - protein, 107 aa, Artificial sequence
  An artificially synthesized peptide sequence
DIVMTQSPLSLPVTPGEPASISCKASQDIDDDMNWYLQKPGQSPQLLIYEATTLVPGVPDRFSGSGSGTDFTLKISRVEAEDVGVYYCLQHDNFPYTFGQGTKLEIK

SEQ ID NO: 56 - protein, 107 aa, Artificial sequence
  An artificially synthesized peptide sequence
EIVLTQSPGTLSLSPGERATLSCKASQDIDDDMNWYQQKPGQAPRLLIYEATTLVPGIPDRFSGSGSGTDFTLTISRLEPEDFAVYYCLQHDNFPYTFGQGTKVEIK

SEQ ID NO: 57 - protein, 107 aa, Artificial sequence
  An artificially synthesized peptide sequence
DIVMTQSPDSLAVSLGERATINCKASQDIDDDMNWYQQKPGQPPKLLIYEATTLVPGVPDRFSGSGSGTDFTLTISSLQAEDVAVYYCLQHDNFPYTFGQGTKLEIK

SEQ ID NO: 58 - protein, 214 aa, Artificial sequence
  An artificially synthesized peptide sequence
ETTLTQSPAFMSATPGDKVTISCKASQDIADDMNWYQQKPGEAAIFIIQEATTLVPGISPRFSGSGYGTDFTLTINNIESEDAAYYFCLQHDNFPYTFGQGTKLEIKRTVAAPSVFIFPPSDEQLKSGTASVVCLLNNFYPREAKVQWKVDNALQSGNSQESVTEQDSKDSTYSLSSTLTLSKADYEKHKVYACEVTHQGLSSPVTKSFNRGEC

SEQ ID NO: 59 - protein, 214 aa, Artificial sequence
  An artificially synthesized peptide sequence
ETTLTQSPAFMSATPGDKVTISCKASQDIDADMNWYQQKPGEAAIFIIQEATTLVPGISPRFSGSGYGTDFTLTINNIESEDAAYYFCLQHDNFPYTFGQGTKLEIKRTVAAPSVFIFPPSDEQLKSGTASVVCLLNNFYPREAKVQWKVDNALQSGNSQESVTEQDSKDSTYSLSSTLTLSKADYEKHKVYACEVTHQGLSSPVTKSFNRGEC

SEQ ID NO: 60 - protein, 214 aa, Artificial sequence
  An artificially synthesized peptide sequence
ETTLTQSPAFMSATPGDKVTISCKASQDIDDAMNWYQQKPGEAAIFIIQEATTLVPGISPRFSGSGYGTDFTLTINNIESEDAAYYFCLQHDNFPYTFGQGTKLEIKRTVAAPSVFIFPPSDEQLKSGTASVVCLLNNFYPREAKVQWKVDNALQSGNSQESVTEQDSKDSTYSLSSTLTLSKADYEKHKVYACEVTHQGLSSPVTKSFNRGEC

SEQ ID NO: 61 - protein, 214 aa, Artificial sequence
  An artificially synthesized peptide sequence
ETTLTQSPAFMSATPGDKVTISCKASQDIDDDMNWYQQKPGEAAIFIIQAATTLVPGISPRFSGSGYGTDFTLTINNIESEDAAYYFCLQHDNFPYTFGQGTKLEIKRTVAAPSVFIFPPSDEQLKSGTASVVCLLNNFYPREAKVQWKVDNALQSGNSQESVTEQDSKDSTYSLSSTLTLSKADYEKHKVYACEVTHQGLSSPVTKSFNRGEC

SEQ ID NO: 62 - protein, 214 aa, Artificial sequence
  An artificially synthesized peptide sequence
ETTLTQSPAFMSATPGDKVTISCKASQDIADAMNWYQQKPGEAAIFIIQEATTLVPGISPRFSGSGYGTDFTLTINNIESEDAAYYFCLQHDNFPYTFGQGTKLEIKRTVAAPSVFIFPPSDEQLKSGTASVVCLLNNFYPREAKVQWKVDNALQSGNSQESVTEQDSKDSTYSLSSTLTLSKADYEKHKVYACEVTHQGLSSPVTKSFNRGEC

SEQ ID NO: 63 - protein, 214 aa, Artificial sequence
  An artificially synthesized peptide sequence
ETTLTQSPAFMSATPGDKVTISCKASQDIADDMNWYQQKPGEAAIFIIQAATTLVPGISPRFSGSGYGTDFTLTINNIESEDAAYYFCLQHDNFPYTFGQGTKLEIKRTVAAPSVFIFPPSDEQLKSGTASVVCLLNNFYPREAKVQWKVDNALQSGNSQESVTEQDSKDSTYSLSSTLTLSKADYEKHKVYACEVTHQGLSSPVTKSFNRGEC

SEQ ID NO: 64 - protein, 214 aa, Artificial sequence
  An artificially synthesized peptide sequence
ETTLTQSPAFMSATPGDKVTISCKASQDIADAMNWYQQKPGEAAIFIIQAATTLVPGISPRFSGSGYGTDFTLTINNIESEDAAYYFCLQHDNFPYTFGQGTKLEIKRTVAAPSVFIFPPSDEQLKSGTASVVCLLNNFYPREAKVQWKVDNALQSGNSQESVTEQDSKDSTYSLSSTLTLSKADYEKHKVYACEVTHQGLSSPVTKSFNRGEC

SEQ ID NO: 65 - protein, 214 aa, Artificial sequence
  An artificially synthesized peptide sequence
ETTLTQSPAFMSATPGDKVTISCKASQDIDDDMNWYQQKPGEAAIFIIQEATTLVPGISPRFSGSGYGTDFTLTINNIESEDAAYYFCLQHANFPYTFGQGTKLEIKRTVAAPSVFIFPPSDEQLKSGTASVVCLLNNFYPREAKVQWKVDNALQSGNSQESVTEQDSKDSTYSLSSTLTLSKADYEKHKVYACEVTHQGLSSPVTKSFNRGEC

SEQ ID NO: 66 - protein, 214 aa, Artificial sequence
  An artificially synthesized peptide sequence
DIQMTQSPSSLSASVGDRVTITCRASQSIDDDLNWYQQKPGKAPKLLIYEASSLQSGVPSRFSGSGSGTDFTLTISSLQPEDFATYYCQQSDSTPYTFGQGTKVEIKRTVAAPSVFIFPPSDEQLKSGTASVVCLLNNFYPREAKVQWKVDNALQSGNSQESVTEQDSKDSTYSLSSTLTLSKADYEKHKVYACEVTHQGLSSPVTKSFNRGEC

SEQ ID NO: 67 - protein, 214 aa, Artificial sequence
  An artificially synthesized peptide sequence
DIQMTQSPSSLSASVGDRVTITCRASQSISSYLNWYQQKPGKAPKLLIYAASSLQSGVPSRFSGSGSGTDFTLTISSLQPEDFATYYCQQSYSTPYTFGQGTKVEIKRTVAAPSVFIFPPSDEQLKSGTASVVCLLNNFYPREAKVQWKVDNALQSGNSQESVTEQDSKDSTYSLSSTLTLSKADYEKHKVYACEVTHQGLSSPVTKSFNRGEC

SEQ ID NO: 68 - protein, 456 aa, Artificial sequence
  An artificially synthesized peptide sequence
QVQLQESGPGLVKPSETLSLTCTVSGGSISSSSYYWGWIRQPPGKGLEWIGSIYYSGSTYYNPSLKSRVTISVDTSKNQFSLKLSSVTAADTAVYYCARVPPYSSSSYYYYYYYMDVWGKGTTVTVSSASTKGPSVFPLAPSSKSTSGGTAALGCLVKDYFPEPVTVSWNSGALTSGVHTFPAVLQSSGLYSLSSVVTVPSSSLGTQTYICNVNHKPSNTKVDKKVEPKSCDKTHTCPPCPAPELLGGPSVFLFPPKPKDTLMISRTPEVTCVVVDVSHEDPEVKFNWYVDGVEVHNAKTKPREEQYNSTYRVVSVLTVLHQDWLNGKEYKCKVSNKALPAPIEKTISKAKGQPREPQVYTLPPSRDELTKNQVSLTCLVKGFYPSDIAVEWESNGQPENNYKTTPPVLDSDGSFFLYSKLTVDKSRWQQGNVFSCSVMHEALHNHYTQKSLSLSP

SEQ ID NO: 69 - protein, 452 aa, Artificial sequence
  An artificially synthesized peptide sequence
EVQLVESGGGLVQPGGSLRLSCAASGFTFSSYAMSWVRQAPGKGLEWVSAISGSGGSTYYADSVKGRFTISRDNSKNTLYLQMNSLRAEDTAVYYCAKAPGIQLWLRPSYFDYWGQGTLVTVSSASTKGPSVFPLAPSSKSTSGGTAALGCLVKDYFPEPVTVSWNSGALTSGVHTFPAVLQSSGLYSLSSVVTVPSSSLGTQTYICNVNHKPSNTKVDKKVEPKSCDKTHTCPPCPAPELLGGPSVFLFPPKPKDTLMISRTPEVTCVVVDVSHEDPEVKFNWYVDGVEVHNAKTKPREEQYNSTYRVVSVLTVLHQDWLNGKEYKCKVSNKALPAPIEKTISKAKGQPREPQVYTLPPSRDELTKNQVSLTCLVKGFYPSDIAVEWESNGQPENNYKTTPPVLDSDGSFFLYSKLTVDKSRWQQGNVFSCSVMHEALHNHYTQKSLSLSP

SEQ ID NO: 70 - protein, 447 aa, Artificial sequence
  An artificially synthesized peptide sequence
QVQLQESGPGLVKPWETLSLTCTVAGDSIKYSSDYWGWVRQSPGKGLEWIGSSYLSGTTQYNPSLKSRVTMSVDTSKNQFSLRLSSVTAADTAVYYCARHRGPTGVDQWGQGTLVTVSSASTKGPSVFPLAPSSKSTSGGTAALGCLVKDYFPEPVTVSWNSGALTSGVHTFPAVLQSSGLYSLSSVVTVPSSSLGTQTYICNVNHKPSNTKVDKKVEPKSCDKTHTCPPCPAPELLGGPSVFLFPPKPKDTLMISRTPEVTCVVVDVSHEDPEVKFNWYVDGVEVHNAKTKPREEQYNSTYRVVSVLTVLHQDWLNGKEYKCKVSNKALPAPIEKTISKAKGQPREPQVYTLPPSRDELTKNQVSLTCLVKGFYPSDIAVEWESNGQPENNYKTTPPVLDSDGSFFLYSKLTVDKSRWQQGNVFSCSVMHEALHNHYTQKSLSLSP

SEQ ID NO: 71 - protein, 449 aa, Artificial sequence
  An artificially synthesized peptide sequence
EVQLVQSGGGLVQPGRSLTLSCVGYGFTFHENDMHWLRQPLGKGLEWVSHIGWNNNRVAYADSVKGRFAVSRDNAKNSLFLHMNSLRPDDTALYYCAKDLGNPIYDVFDVWGQGTMVTVSSASTKGPSVFPLAPSSKSTSGGTAALGCLVKDYFPEPVTVSWNSGALTSGVHTFPAVLQSSGLYSLSSVVTVPSSSLGTQTYICNVNHKPSNTKVDKKVEPKSCDKTHTCPPCPAPELLGGPSVFLFPPKPKDTLMISRTPEVTCVVVDVSHEDPEVKFNWYVDGVEVHNAKTKPREEQYNSTYRVVSVLTVLHQDWLNGKEYKCKVSNKALPAPIEKTISKAKGQPREPQVYTLPPSRDELTKNQVSLTCLVKGFYPSDIAVEWESNGQPENNYKTTPPVLDSDGSFFLYSKLTVDKSRWQQGNVFSCSVMHEALHNHYTQKSLSLSP

SEQ ID NO: 72 - protein, 452 aa, Artificial sequence
  An artificially synthesized peptide sequence
QPALAQMQLVESGGGLVQPGRSLRLSCAASGFTFDDYAMHWVRQAPGKGLEWVSGISWNSGSIGYADSVKGRFTISRDNAKNSLYLQMNSLRAEDTALYYCAREGVLGDAFDIWGQGTMVTVSSASTKGPSVFPLAPSSKSTSGGTAALGCLVKDYFPEPVTVSWNSGALTSGVHTFPAVLQSSGLYSLSSVVTVPSSSLGTQTYICNVNHKPSNTKVDKKVEPKSCDKTHTCPPCPAPELLGGPSVFLFPPKPKDTLMISRTPEVTCVVVDVSHEDPEVKFNWYVDGVEVHNAKTKPREEQYNSTYRVVSVLTVLHQDWLNGKEYKCKVSNKALPAPIEKTISKAKGQPREPQVYTLPPSRDELTKNQVSLTCLVKGFYPSDIAVEWESNGQPENNYKTTPPVLDSDGSFFLYSKLTVDKSRWQQGNVFSCSVMHEALHNHYTQKSLSLSP

SEQ ID NO: 73 - protein, 454 aa, Artificial sequence
  An artificially synthesized peptide sequence
QVQLQQSGPGLVKPSQTLSLTCAISGDSVSSNSAAWNWIRQSPSRGLEWLGRTYYRSKWYNDYAVSVKSRITINPDTSKNQFSLQLNSVTPEDTAVYYCARRVRSGSYYYYGMDVWGQGTTVTVSSASTKGPSVFPLAPSSKSTSGGTAALGCLVKDYFPEPVTVSWNSGALTSGVHTFPAVLQSSGLYSLSSVVTVPSSSLGTQTYICNVNHKPSNTKVDKKVEPKSCDKTHTCPPCPAPELLGGPSVFLFPPKPKDTLMISRTPEVTCVVVDVSHEDPEVKFNWYVDGVEVHNAKTKPREEQYNSTYRVVSVLTVLHQDWLNGKEYKCKVSNKALPAPIEKTISKAKGQPREPQVYTLPPSRDELTKNQVSLTCLVKGFYPSDIAVEWESNGQPENNYKTTPPVLDSDGSFFLYSKLTVDKSRWQQGNVFSCSVMHEALHNHYTQKSLSLSP

SEQ ID NO: 74 - protein, 450 aa, Artificial sequence
  An artificially synthesized peptide sequence
QVQLQESGPGLVKPSQTLSLTCAISGDSVSSNSAAWNWIRQSPSRGLEWLGRTYYRSKWYNDYAVSVKSRITIIPDTSKNQFSLQLNSVTPEDTAVYYCARKDPRVWAFDIWGQGTMVTVSSASTKGPSVFPLAPSSKSTSGGTAALGCLVKDYFPEPVTVSWNSGALTSGVHTFPAVLQSSGLYSLSSVVTVPSSSLGTQTYICNVNHKPSNTKVDKKVEPKSCDKTHTCPPCPAPELLGGPSVFLFPPKPKDTLMISRTPEVTCVVVDVSHEDPEVKFNWYVDGVEVHNAKTKPREEQYNSTYRVVSVLTVLHQDWLNGKEYKCKVSNKALPAPIEKTISKAKGQPREPQVYTLPPSRDELTKNQVSLTCLVKGFYPSDIAVEWESNGQPENNYKTTPPVLDSDGSFFLYSKLTVDKSRWQQGNVFSCSVMHEALHNHYTQKSLSLSP

SEQ ID NO: 75 - protein, 449 aa, Artificial sequence
  An artificially synthesized peptide sequence
EVQLVQSGAEVKKPGSSVKVSCKASGGTFSSYAISWVRQAPGQGLEWMGRIIPVLAIANYAQKFQGRVTITADKSTHTAYMELSSLRSGDTAVYYCARDSGYSAGYGGDYWGQGTLVTVSSASTKGPSVFPLAPSSKSTSGGTAALGCLVKDYFPEPVTVSWNSGALTSGVHTFPAVLQSSGLYSLSSVVTVPSSSLGTQTYICNVNHKPSNTKVDKKVEPKSCDKTHTCPPCPAPELLGGPSVFLFPPKPKDTLMISRTPEVTCVVVDVSHEDPEVKFNWYVDGVEVHNAKTKPREEQYNSTYRVVSVLTVLHQDWLNGKEYKCKVSNKALPAPIEKTISKAKGQPREPQVYTLPPSRDELTKNQVSLTCLVKGFYPSDIAVEWESNGQPENNYKTTPPVLDSDGSFFLYSKLTVDKSRWQQGNVFSCSVMHEALHNHYTQKSLSLSP

SEQ ID NO: 76 - protein, 447 aa, Artificial sequence
  An artificially synthesized peptide sequence
EVQLVESGGDLVQPGGSLRLSCAASGFTFKTYWMNWVRQAPGKGLEWVANIRADGGQMYYADSVKGRFTISRDNAKDSLYLQMISLRPEDTALYYCARDPFASGGLDQWGQGTMVTVSSASTKGPSVFPLAPSSKSTSGGTAALGCLVKDYFPEPVTVSWNSGALTSGVHTFPAVLQSSGLYSLSSVVTVPSSSLGTQTYICNVNHKPSNTKVDKKVEPKSCDKTHTCPPCPAPELLGGPSVFLFPPKPKDTLMISRTPEVTCVVVDVSHEDPEVKFNWYVDGVEVHNAKTKPREEQYNSTYRVVSVLTVLHQDWLNGKEYKCKVSNKALPAPIEKTISKAKGQPREPQVYTLPPSRDELTKNQVSLTCLVKGFYPSDIAVEWESNGQPENNYKTTPPVLDSDGSFFLYSKLTVDKSRWQQGNVFSCSVMHEALHNHYTQKSLSLSP

SEQ ID NO: 77 - protein, 450 aa, Artificial sequence
  An artificially synthesized peptide sequence
EVQLVESGGGVVQPGRSLRLSCAASGFTFSSYGMEWVRQAPGKGLEWVALISHDGNNKYYADSVEGRFTISRDNSRNTLYLQMNSLRAEDTAVYYCAKDRVRYFDSYGMDVWGHGTTVTVSSASTKGPSVFPLAPSSKSTSGGTAALGCLVKDYFPEPVTVSWNSGALTSGVHTFPAVLQSSGLYSLSSVVTVPSSSLGTQTYICNVNHKPSNTKVDKKVEPKSCDKTHTCPPCPAPELLGGPSVFLFPPKPKDTLMISRTPEVTCVVVDVSHEDPEVKFNWYVDGVEVHNAKTKPREEQYNSTYRVVSVLTVLHQDWLNGKEYKCKVSNKALPAPIEKTISKAKGQPREPQVYTLPPSRDELTKNQVSLTCLVKGFYPSDIAVEWESNGQPENNYKTTPPVLDSDGSFFLYSKLTVDKSRWQQGNVFSCSVMHEALHNHYTQKSLSLSP

SEQ ID NO: 78 - protein, 449 aa, Artificial sequence
  An artificially synthesized peptide sequence
EVQLVQSGAEVKKPGESLRISCKGSGYSFTSFWINWVRQMPGKGLEWMGNIDPSDSYTNYSPSFQGHVAISADKSISTAYLHWNSLKASDTAMYYCARHRYLGQLAPFDPWGQGTLVTVSSASTKGPSVFPLAPSSKSTSGGTAALGCLVKDYFPEPVTVSWNSGALTSGVHTFPAVLQSSGLYSLSSVVTVPSSSLGTQTYICNVNHKPSNTKVDKKVEPKSCDKTHTCPPCPAPELLGGPSVFLFPPKPKDTLMISRTPEVTCVVVDVSHEDPEVKFNWYVDGVEVHNAKTKPREEQYNSTYRVVSVLTVLHQDWLNGKEYKCKVSNKALPAPIEKTISKAKGQPREPQVYTLPPSRDELTKNQVSLTCLVKGFYPSDIAVEWESNGQPENNYKTTPPVLDSDGSFFLYSKLTVDKSRWQQGNVFSCSVMHEALHNHYTQKSLSLSP

SEQ ID NO: 79 - protein, 214 aa, Artificial sequence
  An artificially synthesized peptide sequence
DIQMTQSPSSLSASVGDRVTITCRASQSIEDDLAWYQQKPGKAPKLLIYEASSLQSGVPSRFSGSGSGTDFTLTISSLQPEDFATYYCQQRDNYPLTFGQGTKVEIKRTVAAPSVFIFPPSDEQLKSGTASVVCLLNNFYPREAKVQWKVDNALQSGNSQESVTEQDSKDSTYSLSSTLTLSKADYEKHKVYACEVTHQGLSSPVTKSFNRGEC

SEQ ID NO: 80 - protein, 214 aa, Artificial sequence
  An artificially synthesized peptide sequence
DIQMTQSPSSLSASVGDRVTITCRASQSIEDDLAWYQQKPGKAPKLLIYHASTLQSGVPSRFSGSGSGTDFTLTISSLQPEDFATYYCQQSDSSPLTFGQGTKVEIKRTVAAPSVFIFPPSDEQLKSGTASVVCLLNNFYPREAKVQWKVDNALQSGNSQESVTEQDSKDSTYSLSSTLTLSKADYEKHKVYACEVTHQGLSSPVTKSFNRGEC

SEQ ID NO: 81 - protein, 214 aa, Artificial sequence
  An artificially synthesized peptide sequence
DIQMTQSPSSLSASVGDRVTITCRASQSIEDDLAWYQQKPGKAPKLLIYEASSLQSGVPSRFSGSGSGTDFTLTISSLQPEDFATYYCQQSSNYPLTFGQGTKVEIKRTVAAPSVFIFPPSDEQLKSGTASVVCLLNNFYPREAKVQWKVDNALQSGNSQESVTEQDSKDSTYSLSSTLTLSKADYEKHKVYACEVTHQGLSSPVTKSFNRGEC

SEQ ID NO: 82 - protein, 214 aa, Artificial sequence
  An artificially synthesized peptide sequence
DIQMTQSPSSLSASVGDRVTITCRASQSIEDDLAWYQQKPGKAPKLLIYEASSLQSGVPSRFSGSGSGTDFTLTISSLQPEDFATYYCQQSDGYPYTFGQGTKVEIKRTVAAPSVFIFPPSDEQLKSGTASVVCLLNNFYPREAKVQWKVDNALQSGNSQESVTEQDSKDSTYSLSSTLTLSKADYEKHKVYACEVTHQGLSSPVTKSFNRGEC

SEQ ID NO: 83 - protein, 214 aa, Artificial sequence
  An artificially synthesized peptide sequence
DIQMTQSPSSLSASVGDRVTITCRASQSIEDDLNWYQQKPGKAPKLLIYEASNLQSGVPSRFSGSGSGTDFTLTISSLQPEDFATYYCQQHSSSPYTFGQGTKVEIKRTVAAPSVFIFPPSDEQLKSGTASVVCLLNNFYPREAKVQWKVDNALQSGNSQESVTEQDSKDSTYSLSSTLTLSKADYEKHKVYACEVTHQGLSSPVTKSFNRGEC

SEQ ID NO: 84 - protein, 214 aa, Artificial sequence
  An artificially synthesized peptide sequence
DIQMTQSPSSLSASVGDRVTITCRASQSIEDDLAWYQQKPGKAPKLLIYEASNLQSGVPSRFSGSGSGTDFTLTISSLQPEDFATYYCQQYDSYPYTFGQGTKVEIKRTVAAPSVFIFPPSDEQLKSGTASVVCLLNNFYPREAKVQWKVDNALQSGNSQESVTEQDSKDSTYSLSSTLTLSKADYEKHKVYACEVTHQGLSSPVTKSFNRGEC

SEQ ID NO: 85 - protein, 214 aa, Artificial sequence
  An artificially synthesized peptide sequence
DIQMTQSPSSLSASVGDRVTITCRASQSISDDLAWYQQKPGKAPKLLIYHASHLQSGVPSRFSGSGSGTDFTLTISSLQPEDFATYYCQQYDNSPLTFGQGTKVEIKRTVAAPSVFIFPPSDEQLKSGTASVVCLLNNFYPREAKVQWKVDNALQSGNSQESVTEQDSKDSTYSLSSTLTLSKADYEKHKVYACEVTHQGLSSPVTKSFNRGEC

SEQ ID NO: 86 - protein, 214 aa, Artificial sequence
  An artificially synthesized peptide sequence
DIQMTQSPSSLSASVGDRVTITCRASQSISDDLAWYQQKPGKAPKLLIYHASNLQSGVPSRFSGSGSGTDFTLTISSLQPEDFATYYCQQYDNYPYTFGQGTKVEIKRTVAAPSVFIFPPSDEQLKSGTASVVCLLNNFYPREAKVQWKVDNALQSGNSQESVTEQDSKDSTYSLSSTLTLSKADYEKHKVYACEVTHQGLSSPVTKSFNRGEC

SEQ ID NO: 87 - protein, 214 aa, Artificial sequence
  An artificially synthesized peptide sequence
DIQMTQSPSSLSASVGDRVTITCRASQSIEDDLNWYQQKPGKAPKLLIYEASSLQSGVPSRFSGSGSGTDFTLTISSLQPEDFATYYCQQRDSSPYTFGQGTKVEIKRTVAAPSVFIFPPSDEQLKSGTASVVCLLNNFYPREAKVQWKVDNALQSGNSQESVTEQDSKDSTYSLSSTLTLSKADYEKHKVYACEVTHQGLSSPVTKSFNRGEC

SEQ ID NO: 88 - protein, 214 aa, Artificial sequence
  An artificially synthesized peptide sequence
DIQMTQSPSSLSASVGDRVTITCRASQSIEDDLNWYQQKPGKAPKLLIYEASSLQSGVPSRFSGSGSGTDFTLTISSLQPEDFATYYCQQSNDYPYTFGQGTKVEIKRTVAAPSVFIFPPSDEQLKSGTASVVCLLNNFYPREAKVQWKVDNALQSGNSQESVTEQDSKDSTYSLSSTLTLSKADYEKHKVYACEVTHQGLSSPVTKSFNRGEC

SEQ ID NO: 89 - protein, 214 aa, Artificial sequence
  An artificially synthesized peptide sequence
DIQMTQSPSSLSASVGDRVTITCRASQSIEDDLAWYQQKPGKAPKLLIYEASSLQSGVPSRFSGSGSGTDFTLTISSLQPEDFATYYCQQHDNYPYTFGQGTKVEIKRTVAAPSVFIFPPSDEQLKSGTASVVCLLNNFYPREAKVQWKVDNALQSGNSQESVTEQDSKDSTYSLSSTLTLSKADYEKHKVYACEVTHQGLSSPVTKSFNRGEC

SEQ ID NO: 90 - protein, 455 aa, Artificial sequence
  An artificially synthesized peptide sequence
QVQLVQSGAEVKKPGSSVKVSCKASGGTFSSYAISWVRQAPGQGLEWMGGIIPIFGTANYAQKFQGRVTITADESTSTAYMELSSLRSEDTAVYYCARAAFLEWPIWGSEYFQHWGQGTLVTVSSASTKGPSVFPLAPSSKSTSGGTAALGCLVKDYFPEPVTVSWNSGALTSGVHTFPAVLQSSGLYSLSSVVTVPSSSLGTQTYICNVNHKPSNTKVDKKVEPKSCDKTHTCPPCPAPELLGGPSVFLFPPKPKDTLMISRTPEVTCVVVDVSHEDPEVKFNWYVDGVEVHNAKTKPREEQYNSTYRVVSVLTVLHQDWLNGKEYKCKVSNKALPAPIEKTISKAKGQPREPQVYTLPPSRDELTKNQVSLTCLVKGFYPSDIAVEWESNGQPENNYKTTPPVLDSDGSFFLYSKLTVDKSRWQQGNVFSCSVMHEALHNHYTQKSLSLSPGK

SEQ ID NO: 91 - protein, 214 aa, Artificial sequence
  An artificially synthesized peptide sequence
DIQMTQSPSSLSASVGDRVTITCRASQSIEDDLAWYQQKPGKAPKLLIYHASSLQSGVPSRFSGSGSGTDFTLTISSLQPEDFATYYCQQRDSYPLTFGQGTKVEIKRTVAAPSVFIFPPSDEQLKSGTASVVCLLNNFYPREAKVQWKVDNALQSGNSQESVTEQDSKDSTYSLSSTLTLSKADYEKHKVYACEVTHQGLSSPVTKSFNRGEC

SEQ ID NO: 92 - protein, 453 aa, Artificial sequence
  An artificially synthesized peptide sequence
QVQLVQSGAEVKKPGASVKVSCKASGYTFTSYGISWVRQAPGQGLEWMGWISAYNGNTNYAQKLQGRVTMTTDTSTSTAYMELRSLRSDDTAVYYCARATYYYDSSAPAFDIWGQGTMVTVSSASTKGPSVFPLAPSSKSTSGGTAALGCLVKDYFPEPVTVSWNSGALTSGVHTFPAVLQSSGLYSLSSVVTVPSSSLGTQTYICNVNHKPSNTKVDKKVEPKSCDKTHTCPPCPAPELLGGPSVFLFPPKPKDTLMISRTPEVTCVVVDVSHEDPEVKFNWYVDGVEVHNAKTKPREEQYNSTYRVVSVLTVLHQDWLNGKEYKCKVSNKALPAPIEKTISKAKGQPREPQVYTLPPSRDELTKNQVSLTCLVKGFYPSDIAVEWESNGQPENNYKTTPPVLDSDGSFFLYSKLTVDKSRWQQGNVFSCSVMHEALHNHYTQKSLSLSPGK

SEQ ID NO: 93 - protein, 214 aa, Artificial sequence
  An artificially synthesized peptide sequence
DIQMTQSPSSLSASVGDRVTITCRASQSIEDDLAWYQQKPGKAPKLLIYEASTLQSGVPSRFSGSGSGTDFTLTISSLQPEDFATYYCQQHDDSPLTFGQGTKVEIKRTVAAPSVFIFPPSDEQLKSGTASVVCLLNNFYPREAKVQWKVDNALQSGNSQESVTEQDSKDSTYSLSSTLTLSKADYEKHKVYACEVTHQGLSSPVTKSFNRGEC

SEQ ID NO: 94 - protein, 454 aa, Artificial sequence
  An artificially synthesized peptide sequence
EVQLVQSGAEVKKPGSSVKVSCKASGGTFSSYAISWVRQAPGQGLEWMGGIIPIFGTANYAQKFQGRVTITADESTSTAYMELSSLRSEDTAVYYCARDRGSGFNWGNYAFDIWGQGFSVTVSSASTKGPSVFPLAPSSKSTSGGTAALGCLVKDYFPEPVTVSWNSGALTSGVHTFPAVLQSSGLYSLSSVVTVPSSSLGTQTYICNVNHKPSNTKVDKKVEPKSCDKTHTCPPCPAPELLGGPSVFLFPPKPKDTLMISRTPEVTCVVVDVSHEDPEVKFNWYVDGVEVHNAKTKPREEQYNSTYRVVSVLTVLHQDWLNGKEYKCKVSNKALPAPIEKTISKAKGQPREPQVYTLPPSRDELTKNQVSLTCLVKGFYPSDIAVEWESNGQPENNYKTTPPVLDSDGSFFLYSKLTVDKSRWQQGNVFSCSVMHEALHNHYTQKSLSLSPGK

SEQ ID NO: 95 - protein, 214 aa, Artificial sequence
  An artificially synthesized peptide sequence
DIQMTQSPSSLSASVGDRVTITCRASQSIEDDLAWYQQKPGKAPKLLIYEASNLQSGVPSRFSGSGSGTDFTLTISSLQPEDFATYYCQQYDRYPYTFGQGTKVEIKRTVAAPSVFIFPPSDEQLKSGTASVVCLLNNFYPREAKVQWKVDNALQSGNSQESVTEQDSKDSTYSLSSTLTLSKADYEKHKVYACEVTHQGLSSPVTKSFNRGEC

SEQ ID NO: 96 - protein, 449 aa, Artificial sequence
  An artificially synthesized peptide sequence
QVQLQESGPGLVRPSQTLSLTCTVSGYSITSDHAWSWVRQPPGRGLEWIGYISYSGITTYNPSLKSRVTMLRDTSKNQFSLRLSSVTAADTAVYYCARSLARTTAMDYWGQGSLVTVSSASTKGPSVFPLAPSSKSTSGGTAALGCLVKDYFPEPVTVSWNSGALTSGVHTFPAVLQSSGLYSLSSVVTVPSSSLGTQTYICNVNHKPSNTKVDKKVEPKSCDKTHTCPPCPAPELLGGPSVFLFPPKPKDTLMISRTPEVTCVVVDVSHEDPEVKFNWYVDGVEVHNAKTKPREEQYNSTYRVVSVLTVLHQDWLNGKEYKCKVSNKALPAPIEKTISKAKGQPREPQVYTLPPSRDELTKNQVSLTCLVKGFYPSDIAVEWESNGQPENNYKTTPPVLDSDGSFFLYSKLTVDKSRWQQGNVFSCSVMHEALHNHYTQKSLSLSPGK

SEQ ID NO: 97 - protein, 214 aa, Artificial sequence [sequence omitted]

SEQ ID NO: 98 - protein, 449 aa, Artificial sequence; identical to SEQ ID NO: 9
  An artificially synthesized peptide sequence

SEQ ID NO: 99 - protein, 217 aa, Artificial sequence
  An artificially synthesized peptide sequence
QSVLTQPPSVSGAPGQRVTISCTGSRSNMGAGYDVHWYQLLPGAAPKLLISHNTHRPSGVPDRFSGSKSGASASLAITGLQAEDEADYYCQSHDSSLSAVVFGGGTKLTVLSQPKAAPSVTLFPPSSEELQANKATLVCLISDFYPGAVTVAWKADSSPVKAGVETTTPSKQSNNKYAASSYLSLTPEQWKSHRSYSCQVTHEGSTVEKTVAPTECS

SEQ ID NO: 100 - protein, 455 aa, Artificial sequence
  An artificially synthesized peptide sequence
QVQLVQSGAEVKKPGSSVKVSCKASGGTFSSYAISWVRQAPGQGLEWMGGIIPIFGTANYAQKFQGRVTITADESTSTAYMELSSLRSEDTAVYYCARERDYYDSSGYYDAFDIWGQGTMVTVSSASTKGPSVFPLAPSSKSTSGGTAALGCLVKDYFPEPVTVSWNSGALTSGVHTFPAVLQSSGLYSLSSVVTVPSSSLGTQTYICNVNHKPSNTKVDKKVEPKSCDKTHTCPPCPAPELLGGPSVFLFPPKPKDTLMISRTPEVTCVVVDVSHEDPEVKFNWYVDGVEVHNAKTKPREEQYNSTYRVVSVLTVLHQDWLNGKEYKCKVSNKALPAPIEKTISKAKGQPREPQVYTLPPSRDELTKNQVSLTCLVKGFYPSDIAVEWESNGQPENNYKTTPPVLDSDGSFFLYSKLTVDKSRWQQGNVFSCSVMHEALHNHYTQKSLSLSPGK

SEQ ID NO: 101 - protein, 214 aa, Artificial sequence
  An artificially synthesized peptide sequence
ETTVTQSPSFLSASVGDRVTITCITTTDIDDDMNWFQQEPGKAPKLLISEGNILRPGVPSRFSSSGYGTDFTLTISKLQPEDFATYYCLQSDNLPFTFGQGTKLEIKRTVAAPSVFIFPPSDEQLKSGTASVVCLLNNFYPREAKVQWKVDNALQSGNSQESVTEQDSKDSTYSLSSTLTLSKADYEKHKVYACEVTHQGLSSPVTKSFNRGEC

SEQ ID NO: 102 - protein, 449 aa, Artificial sequence
  An artificially synthesized peptide sequence
QVQLQESGPGLVKPSETLSLTCAVSGYSISDDQAWSWVRQPPGEGLEWIGYISYSGITNYNPSLKGRVTISRDTSKNQFSLKLSSVTAADTAAYYCARSLARTTAMDYWGEGTLVTVSSASTKGPSVFPLAPSSKSTSGGTAALGCLVKDYFPEPVTVSWNSGALTSGVHTFPAVLQSSGLYSLSSVVTVPSSSLGTQTYICNVNHKPSNTKVDKKVEPKSCDKTHTCPPCPAPELLGGPSVFLFPPKPKDTLMISRTPEVTCVVVDVSHEDPEVKFNWYVDGVEVHNAKTKPREEQYNSTYRVVSVLTVLHQDWLNGKEYKCKVSNKALPAPIEKTISKAKGQPREPQVYTLPPSRDELTKNQVSLTCLVKGFYPSDIAVEWESNGQPENNYKTTPPVLDSDGSFFLYSKLTVDKSRWQQGNVFSCSVMHEALHNHYTQKSLSLSPGK

SEQ ID NO: 103 - protein, 214 aa, Artificial sequence; identical to SEQ ID NO: 39
  An artificially synthesized peptide sequence

SEQ ID NO: 104 - protein, 213 aa, Artificial sequence
  An artificially synthesized peptide sequence
EIVLTQSPATLSLSPGERATLSCRASQSVSSYLAWYQQKPGQAPRLLIFDASNRAAGIPARFSGSGSGTDFTLTISSLEPEDFAVYYCQQFDKWVTFGGGTTVEIRRTVAAPSVFIFPPSDEQLKSGTASVVCLLNNFYPREAKVQWKVDNALQSGNSQESVTEQDSKDSTYSLSSTLTLSKADYEKHKVYACEVTHQGLSSPVTKSFNRGEC

SEQ ID NO: 105 - protein, 454 aa, Artificial sequence
  An artificially synthesized peptide sequence
EVQLVESGGGLVQPGGSLRLSCAASGFTFSSYEMNWVRQAPGKGLEWVSYISSSGSTIYYADSVKGRFTISRDNAKNSLYLQMNSLRAEDTAVYYCARDAPYYYDSSGYTDAFDIWGQGTMVTVSSASTKGPSVFPLAPSSKSTSGGTAALGCLVKDYFPEPVTVSWNSGALTSGVHTFPAVLQSSGLYSLSSVVTVPSSSLGTQTYICNVNHKPSNTKVDKKVEPKSCDKTHTCPPCPAPELLGGPSVFLFPPKPKDTLMISRTPEVTCVVVDVSHEDPEVKFNWYVDGVEVHNAKTKPREEQYNSTYRVVSVLTVLHQDWLNGKEYKCKVSNKALPAPIEKTISKAKGQPREPQVYTLPPSRDELTKNQVSLTCLVKGFYPSDIAVEWESNGQPENNYKTTPPVLDSDGSFFLYSKLTVDKSRWQQGNVFSCSVMHEALHNHYTQKSLSLSP

SEQ ID NO: 106 - protein, 443 aa, Artificial sequence
  An artificially synthesized peptide sequence
QVQLVQSGAEVKKPGASVKVSCKASGYTFTDYEMHWVRQAPGQGLEWMGALDPKTGDTAYSQKFKGRVTLTADKSTSTAYMELSSLTSEDTAVYYCTRFYSYTYWGQGTLVTVSSASTKGPSVFPLAPSSKSTSGGTAALGCLVKDYFPEPVTVSWNSGALTSGVHTFPAVLQSSGLYSLSSVVTVPSSSLGTQTYICNVNHKPSNTKVDKKVEPKSCDKTHTCPPCPAPELLGGPSVFLFPPKPKDTLMISRTPEVTCVVVDVSHEDPEVKFNWYVDGVEVHNAKTKPREEQYNSTYRVVSVLTVLHQDWLNGKEYKCKVSNKALPAPIEKTISKAKGQPREPQVYTLPPSRDELTKNQVSLTCLVKGFYPSDIAVEWESNGQPENNYKTTPPVLDSDGSFFLYSKLTVDKSRWQQGNVFSCSVMHEALHNHYTQKSLSLSP

SEQ ID NO: 107 - protein, 219 aa, Artificial sequence
  An artificially synthesized peptide sequence
DVVMTQSPLSLPVTPGEPASISCRSSQSLVHSNRNTYLHWYLQKPGQSPQLLIYKVSNRFSGVPDRFSGSGSGTDFTLKISRVEAEDVGVYYCSQNTHVPPTFGQGTKLEIKRTVAAPSVFIFPPSDEQLKSGTASVVCLLNNFYPREAKVQWKVDNALQSGNSQESVTEQDSKDSTYSLSSTLTLSKADYEKHKVYACEVTHQGLSSPVTKSFNRGEC

SEQ ID NO: 108 - protein, 454 aa, Artificial sequence
  An artificially synthesized peptide sequence
EVQLVESGGGLVQPGGSLRLSCAASGFTFSSYEMNWVRQAPGKGLEWVSYISSSGSTIYYAASVKGRFTISRDNAKNSLYLQMNSLRAEDTAVYYCARDAPYYYDSSGYTDAFDIWGQGTMVTVSSASTKGPSVFPLAPSSKSTSGGTAALGCLVKDYFPEPVTVSWNSGALTSGVHTFPAVLQSSGLYSLSSVVTVPSSSLGTQTYICNVNHKPSNTKVDKKVEPKSCDKTHTCPPCPAPELLGGPSVFLFPPKPKDTLMISRTPEVTCVVVDVSHEDPEVKFNWYVDGVEVHNAKTKPREEQYNSTYRVVSVLTVLHQDWLNGKEYKCKVSNKALPAPIEKTISKAKGQPREPQVYTLPPSRDELTKNQVSLTCLVKGFYPSDIAVEWESNGQPENNYKTTPPVLDSDGSFFLYSKLTVDKSRWQQGNVFSCSVMHEALHNHYTQKSLSLSP

SEQ ID NO: 109 - protein, 454 aa, Artificial sequence
  An artificially synthesized peptide sequence
EVQLVESGGGLVQPGGSLRLSCAASGFTFSSYEMNWVRQAPGKGLEWVSYISSSGSTIYYADSVKGRFTISRDNAKNSLYLQMNSLRAEDTAVYYCARAAPYYYDSSGYTDAFDIWGQGTMVTVSSASTKGPSVFPLAPSSKSTSGGTAALGCLVKDYFPEPVTVSWNSGALTSGVHTFPAVLQSSGLYSLSSVVTVPSSSLGTQTYICNVNHKPSNTKVDKKVEPKSCDKTHTCPPCPAPELLGGPSVFLFPPKPKDTLMISRTPEVTCVVVDVSHEDPEVKFNWYVDGVEVHNAKTKPREEQYNSTYRVVSVLTVLHQDWLNGKEYKCKVSNKALPAPIEKTISKAKGQPREPQVYTLPPSRDELTKNQVSLTCLVKGFYPSDIAVEWESNGQPENNYKTTPPVLDSDGSFFLYSKLTVDKSRWQQGNVFSCSVMHEALHNHYTQKSLSLSP

SEQ ID NO: 110 - protein, 454 aa, Artificial sequence
  An artificially synthesized peptide sequence
EVQLVESGGGLVQPGGSLRLSCAASGFTFSSYEMNWVRQAPGKGLEWVSYISSSGSTIYYADSVKGRFTISRDNAKNSLYLQMNSLRAEDTAVYYCARDAPYYYASSGYTDAFDIWGQGTMVTVSSASTKGPSVFPLAPSSKSTSGGTAALGCLVKDYFPEPVTVSWNSGALTSGVHTFPAVLQSSGLYSLSSVVTVPSSSLGTQTYICNVNHKPSNTKVDKKVEPKSCDKTHTCPPCPAPELLGGPSVFLFPPKPKDTLMISRTPEVTCVVVDVSHEDPEVKFNWYVDGVEVHNAKTKPREEQYNSTYRVVSVLTVLHQDWLNGKEYKCKVSNKALPAPIEKTISKAKGQPREPQVYTLPPSRDELTKNQVSLTCLVKGFYPSDIAVEWESNGQPENNYKTTPPVLDSDGSFFLYSKLTVDKSRWQQGNVFSCSVMHEALHNHYTQKSLSLSP

SEQ ID NO: 111 - protein, 454 aa, Artificial sequence
  An artificially synthesized peptide sequence
EVQLVESGGGLVQPGGSLRLSCAASGFTFSSYEMNWVRQAPGKGLEWVSYISSSGSTIYYADSVKGRFTISRDNAKNSLYLQMNSLRAEDTAVYYCARDAPYYYDSSGYTAAFDIWGQGTMVTVSSASTKGPSVFPLAPSSKSTSGGTAALGCLVKDYFPEPVTVSWNSGALTSGVHTFPAVLQSSGLYSLSSVVTVPSSSLGTQTYICNVNHKPSNTKVDKKVEPKSCDKTHTCPPCPAPELLGGPSVFLFPPKPKDTLMISRTPEVTCVVVDVSHEDPEVKFNWYVDGVEVHNAKTKPREEQYNSTYRVVSVLTVLHQDWLNGKEYKCKVSNKALPAPIEKTISKAKGQPREPQVYTLPPSRDELTKNQVSLTCLVKGFYPSDIAVEWESNGQPENNYKTTPPVLDSDGSFFLYSKLTVDKSRWQQGNVFSCSVMHEALHNHYTQKSLSLSP

SEQ ID NO: 112 - protein, 454 aa, Artificial sequence
  An artificially synthesized peptide sequence
EVQLVESGGGLVQPGGSLRLSCAASGFTFSSYEMNWVRQAPGKGLEWVSYISSSGSTIYYADSVKGRFTISRDNAKNSLYLQMNSLRAEDTAVYYCARDAPYYYDSSGYTDAFAIWGQGTMVTVSSASTKGPSVFPLAPSSKSTSGGTAALGCLVKDYFPEPVTVSWNSGALTSGVHTFPAVLQSSGLYSLSSVVTVPSSSLGTQTYICNVNHKPSNTKVDKKVEPKSCDKTHTCPPCPAPELLGGPSVFLFPPKPKDTLMISRTPEVTCVVVDVSHEDPEVKFNWYVDGVEVHNAKTKPREEQYNSTYRVVSVLTVLHQDWLNGKEYKCKVSNKALPAPIEKTISKAKGQPREPQVYTLPPSRDELTKNQVSLTCLVKGFYPSDIAVEWESNGQPENNYKTTPPVLDSDGSFFLYSKLTVDKSRWQQGNVFSCSVMHEALHNHYTQKSLSLSP

SEQ ID NO: 113 - protein, 213 aa, Artificial sequence
  An artificially synthesized peptide sequence
EIVLTQSPATLSLSPGERATLSCRASQSVSSYLAWYQQKPGQAPRLLIFAASNRAAGIPARFSGSGSGTDFTLTISSLEPEDFAVYYCQQFDKWVTFGGGTTVEIRRTVAAPSVFIFPPSDEQLKSGTASVVCLLNNFYPREAKVQWKVDNALQSGNSQESVTEQDSKDSTYSLSSTLTLSKADYEKHKVYACEVTHQGLSSPVTKSFNRGEC

SEQ ID NO: 114 - protein, 213 aa, Artificial sequence
  An artificially synthesized peptide sequence
EIVLTQSPATLSLSPGERATLSCRASQSVSSYLAWYQQKPGQAPRLLIFDASNRAAGIPARFSGSGSGTDFTLTISSLEPEDFAVYYCQQFAKWVTFGGGTTVEIRRTVAAPSVFIFPPSDEQLKSGTASVVCLLNNFYPREAKVQWKVDNALQSGNSQESVTEQDSKDSTYSLSSTLTLSKADYEKHKVYACEVTHQGLSSPVTKSFNRGEC

SEQ ID NO: 115 - protein, 453 aa, Artificial sequence
  An artificially synthesized peptide sequence
QVQLVQSGAEVKKPGSSVKVSCKASGGTFSSYAISWVRQAPGQGLEWMGGIIPIFGTANYAQKFQGRVTITADESTSTAYMELSSLRSEDTAVYYCARERDYYDSSGYYDAFDIWGQGTMVTVSSASTKGPSVFPLAPSSKSTSGGTAALGCLVKDYFPEPVTVSWNSGALTSGVHTFPAVLQSSGLYSLSSVVTVPSSSLGTQTYICNVNHKPSNTKVDKKVEPKSCDKTHTCPPCPAPELLGGPSVFLFPPKPKDTLMISRTPEVTCVVVDVSHEDPEVKFNWYVDGVEVHNAKTKPREEQYNSTYRVVSVLTVLHQDWLNGKEYKCKVSNKALPAPIEKTISKAKGQPREPQVYTLPPSRDELTKNQVSLTCLVKGFYPSDIAVEWESNGQPENNYKTTPPVLDSDGSFFLYSKLTVDKSRWQQGNVFSCSVMHEALHWHYTQKSLSLSP

SEQ ID NO: 116 - protein, 449 aa, Artificial sequence
  An artificially synthesized peptide sequence
QVQLVQSGAEVKKPGASVKVSCKASGYTFTSYYMHWVRQAPGQGLEWMGIINPSGGSTSYAQKFQGRVTMTRDTSTSTVYMELSSLRSEDTAVYYCARDDPGGGEYYFDYWGQGTLVTVSSASTKGPSVFPLAPSSKSTSGGTAALGCLVKDYFPEPVTVSWNSGALTSGVHTFPAVLQSSGLYSLSSVVTVPSSSLGTQTYICNVNHKPSNTKVDKKVEPKSCDKTHTCPPCPAPELLGGPSVFLFPPKPKDTLMISRTPEVTCVVVDVSHEDPEVKFNWYVDGVEVHNAKTKPREEQYNSTYRVVSVLTVLHQDWLNGKEYKCKVSNKALPAPIEKTISKAKGQPREPQVYTLPPSRDELTKNQVSLTCLVKGFYPSDIAVEWESNGQPENNYKTTPPVLDSDGSFFLYSKLTVDKSRWQQGNVFSCSVMHEALHWHYTQKSLSLSP

SEQ ID NO: 117 - protein, 447 aa, Artificial sequence
  An artificially synthesized peptide sequence
QVQLQESGPGLVKPSETLSLTCAVSGYSISDDQAWSWVRQPPGEGLEWIGYISYSGITNYNPSLKGRVTISRDTSKNQFSLKLSSVTAADTAAYYCARSLARTTAMDYWGEGTLVTVSSASTKGPSVFPLAPSSKSTSGGTAALGCLVKDYFPEPVTVSWNSGALTSGVHTFPAVLQSSGLYSLSSVVTVPSSSLGTQTYICNVNHKPSNTKVDKKVEPKSCDKTHTCPPCPAPELLGGPSVFLFPPKPKDTLMISRTPEVTCVVVDVSHEDPEVKFNWYVDGVEVHNAKTKPREEQYNSTYRVVSVLTVLHQDWLNGKEYKCKVSNKALPAPIEKTISKAKGQPREPQVYTLPPSRDELTKNQVSLTCLVKGFYPSDIAVEWESNGQPENNYKTTPPVLDSDGSFFLYSKLTVDKSRWQQGNVFSCSVMHEALHWHYTQKSLSLSP

SEQ ID NO: 118 - protein, 458 aa, Artificial sequence
  An artificially synthesized peptide sequence
EVQLVQSGAEVKKPGSSVKVSCKASGGTFSSYAISWVRQAPGQGLEWMGGIIPIFGTANYAQKFQGRVTITADESTSTAYMELSSLRSEDTAVYYCARASIYCSSTSCYEPPYYYYMDVWGKGTMVTVSSASTKGPSVFPLAPSSKSTSGGTAALGCLVKDYFPEPVTVSWNSGALTSGVHTFPAVLQSSGLYSLSSVVTVPSSSLGTQTYICNVNHKPSNTKVDKKVEPKSCDKTHTCPPCPAPELLGGPSVFLFPPKPKDTLMISRTPEVTCVVVDVSHEDPEVKFNWYVDGVEVHNAKTKPREEQYNSTYRVVSVLTVLHQDWLNGKEYKCKVSNKALPAPIEKTISKAKGQPREPQVYTLPPSRDELTKNQVSLTCLVKGFYPSDIAVEWESNGQPENNYKTTPPVLDSDGSFFLYSKLTVDKSRWQQGNVFSCSVMHEALHNHYTQKSLSLSP

SEQ ID NO: 119 - protein, 214 aa, Artificial sequence
  An artificially synthesized peptide sequence
DIQMTQSPSSLSASVGDRVTITCRASQSISSHLAWYQQKPGKAPKLLIYAASHLQSGVPSRFSGSGSGTDFTLTISSLQPEDFATYYCQQSHNYPLTFGQGTKVEIKRTVAAPSVFIFPPSDEQLKSGTASVVCLLNNFYPREAKVQWKVDNALQSGNSQESVTEQDSKDSTYSLSSTLTLSKADYEKHKVYACEVTHQGLSSPVTKSFNRGEC

SEQ ID NO: 120 - protein, 447 aa, Artificial sequence
  An artificially synthesized peptide sequence
QVQLVQSGAEVKKPGSSVKVSCKASGGTFSSYAISWVRQAPGQGLEWMGGIIPIFGTANYAQKFQGRVTITADESTSTAYMELSSLRSEDTAVYYCMINGVWEGGMDVWGQGTTVTVSSASTKGPSVFPLAPSSKSTSGGTAALGCLVKDYFPEPVTVSWNSGALTSGVHTFPAVLQSSGLYSLSSVVTVPSSSLGTQTYICNVNHKPSNTKVDKKVEPKSCDKTHTCPPCPAPELLGGPSVFLFPPKPKDTLMISRTPEVTCVVVDVSHEDPEVKFNWYVDGVEVHNAKTKPREEQYNSTYRVVSVLTVLHQDWLNGKEYKCKVSNKALPAPIEKTISKAKGQPREPQVYTLPPSRDELTKNQVSLTCLVKGFYPSDIAVEWESNGQPENNYKTTPPVLDSDGSFFLYSKLTVDKSRWQQGNVFSCSVMHEALHNHYTQKSLSLSP

SEQ ID NO: 121 - protein, 214 aa, Artificial sequence
  An artificially synthesized peptide sequence
DIQMTQSPSSLSASVGDRVTITCRASQSIHSHLNWYQQKPGKAPKLLIYHASKLQSGVPSRFSGSGSGTDFTLTISSLQPEDFATYYCQQHGNSPLTFGQGTKVEIKRTVAAPSVFIFPPSDEQLKSGTASVVCLLNNFYPREAKVQWKVDNALQSGNSQESVTEQDSKDSTYSLSSTLTLSKADYEKHKVYACEVTHQGLSSPVTKSFNRGEC

SEQ ID NO: 122 - protein, 451 aa, Artificial sequence
  An artificially synthesized peptide sequence
EVQLVQSGGGLVQPGGSLRLSCAASGFTFSNAWMIWVRQAPGKGLEWVGRIKSKVDGGTTDYAAPVKGRFTISRDDSKNTLYLQMDSLKTEDTAVYYCVADVPASNPYGFDYWGQGTLVTVSSASTKGPSVFPLAPSSKSTSGGTAALGCLVKDYFPEPVTVSWNSGALTSGVHTFPAVLQSSGLYSLSSVVTVPSSSLGTQTYICNVNHKPSNTKVDKKVEPKSCDKTHTCPPCPAPELLGGPSVFLFPPKPKDTLMISRTPEVTCVVVDVSHEDPEVKFNWYVDGVEVHNAKTKPREEQYNSTYRVVSVLTVLHQDWLNGKEYKCKVSNKALPAPIEKTISKAKGQPREPQVYTLPPSRDELTKNQVSLTCLVKGFYPSDIAVEWESNGQPENNYKTTPPVLDSDGSFFLYSKLTVDKSRWQQGNVFSCSVMHEALHNHYTQKSLSLSP

SEQ ID NO: 123 - protein, 214 aa, Artificial sequence
  An artificially synthesized peptide sequence
DIQMTQSPSSLSASVGDRVTITCRASQSINSHLNWYQQKPGKAPKLLIYDASHLQSGVPSRFSGSGSGTDFTLTISSLQPEDFATYYCQQHNNYPLTFGQGTKVEIKRTVAAPSVFIFPPSDEQLKSGTASVVCLLNNFYPREAKVQWKVDNALQSGNSQESVTEQDSKDSTYSLSSTLTLSKADYEKHKVYACEVTHQGLSSPVTKSFNRGEC

SEQ ID NO: 124 - protein, 443 aa, Artificial sequence
  An artificially synthesized peptide sequence
QVQLQESGPGLVKPSETLSLTCAVSGYSISDDQAWSWVRQPPGEGLEWIGYISYSGITNYNPSLKGRVTISRDTSKNQFSLKLSSVTAADTAAYYCARSLARTTAMDYWGEGTLVTVSSAKTTPPSVYPLAPGSAAQTNSMVTLGCLVKGYFPEPVTVTWNSGSLSSGVHTFPAVLQSDLYTLSSSVTVPSSTWPSETVTCNVAHPASSTKVDKKIVPRDCGCKPCICTVPEVSSVFIFPPKPKDVLYITLEPKVTCVVVDISKDDPEVQFSWFVDDVEVHTAQTQPREEQFNSTFRSVSELPIMHQDWLNGKEFKCRVNSAAFPAPIEKTISKTKGRPKAPQVYTIPPPKEQMAKDKVSLTCMITDFFPEDITVEWQWNGQPAENYKNTQPIMDTDGSYFVYSKLNVQKSNWEAGNTFTCSVLHEGLKFHHTEKSLSHSPGK

SEQ ID NO: 125 - protein, 214 aa, Artificial sequence
  An artificially synthesized peptide sequence
DIQMTQSPSSLSASVGDSVTITCQASQDISSYLNWYQQKPGKAPELLIYYGSELHSGVPSRFSGSGSGTDFTFTISSLEAEDAATYYCQQGNSLPYTFGQGTKVEIERADAAPTVSIFPPSSEQLTSGGASVVCFLNNFYPKDINVKWKIDGSERQNGVLNSWTDQDSKDSTYSMSSTLTLTKDEYERHNSYTCEATHKTSTSPIVKSFNRNEC

SEQ ID NO: 126 - protein, 443 aa, Artificial sequence
  An artificially synthesized peptide sequence
QVQLQESGPGLVKPSETLSLTCAVSGHSISHDHAWSWVRQPPGEGLEWIGFISYSGITNYNPSLQGRVTISRDNSKNTLYLQMNSLRAEDTAVYYCARSLARTTAMDYWGEGTLVTVSSAKTTPPSVYPLAPGSAAQTNSMVTLGCLVKGYFPEPVTVTWNSGSLSSGVHTFPAVLQSDLYTLSSSVTVPSSTWPSETVTCNVAHPASSTKVDKKIVPRDCGCKPCICTVPEVSSVFIFPPKPKDVLTITLTPKVTCVVVDISKDDPEVQFSWFVDDVEVHTAQTQPREEQFNSTFRSVSELPIMHQDWLNGKEFKCRVNSAAFPAPIEKTISKTKGRPKAPQVYTIPPPKEQMAKDKVSLTCMITDFFPEDITVEWQWNGQPAENYKNTQPIMDTDGSYFVYSKLNVQKSNWEAGNTFTCSVLHEGLHNHHTEKSLSHSPGK

SEQ ID NO: 127 - protein, 214 aa, Artificial sequence
  An artificially synthesized peptide sequence
DIQMTQSPSSLSASVGDSVTITCQASTDISSHLNWYQQKPGKAPELLIYYGSHLLSGVPSRFSGSGSGTDFTFTISSLEAEDAATYYCGQGNRLPYTFGQGTKVEIERADAAPTVSIFPPSSEQLTSGGASVVCFLNNFYPKDINVKWKIDGSERQNGVLNSWTDQDSKDSTYSMSSTLTLTKDEYERHNSYTCEATHKTSTSPIVKSFNRNEC

SEQ ID NO: 128 - protein, 449 aa, Artificial sequence
  An artificially synthesized peptide sequence
QVQLQESGPGLVKPSETLSLTCAVSGHSISHDHAWSWVRQPPGEGLEWIGFISYSGITNYNPSLQGRVTISRDNSKNTLYLQMNSLRAEDTAVYYCARSLARTTAMDYWGEGTLVTVSSAKTTAPSVYPLAPVCGDTTGSSVTLGCLVKGYFPEPVTLTWNSGSLSSGVHTFPAVLQSDLYTLSSSVTVTSSTWPSQSITCNVAHPASSTKVDKKIEPRGPTIKPCPPCKCPAPNLLGGPSVFIFPPKIKDVLMISLSPIVTCVVVDVSEDDPDVQISWFVNNVEVHTAQTQTHREDYNSTLRVVSALPIQHQDWMSGKEFKCKVNNKDLPAPIERTISKPKGSVRAPQVYVLPPPEEEMTKKQVTLTCMVTDFMPEDIYVEWTNNGKTELNYKNTEPVLDSDGSYFMYSKLRVEKKNWVERNSYSCSVVHEGLHNHHTTKSFSRTPGK

SEQ ID NO: 129 - protein, 443 aa, Artificial sequence
  An artificially synthesized peptide sequence
QVQLQESGPGLVKPSETLSLTCAVSGHSISHDHAWSWVRQPPGEGLEWIGFISYSGITNYNPSLQGRVTISRDNSKNTLYLQMNSLRAEDTAVYYCARSLARTTAMDYWGEGTLVTVSSAKTTPPSVYPLAPGSAAQTNSMVTLGCLVKGYFPEPVTVTWNSGSLSSGVHTFPAVLQSDLYTLSSSVTVPSSTWPSETVTCNVAHPASSTKVDKKIVPRDCGCKPCICTVPEVSSVFIFPPKPKDVLYITLEPKVTCVVVDISKDDPEVQFSWFVDDVEVHTAQTQPREEQFNSTFRSVSELPIMHQDWLNGKEFKCRVNSAAFPAPIEKTISKTKGRPKAPQVYTIPPPKEQMAKDKVSLTCMITDFFPEDITVEWQWNGQPAENYKNTQPIMDTDGSYFVYSKLNVQKSNWEAGNTFTCSVLHEGLKFHHTEKSLSHSPGK

SEQ ID NO: 130 - protein, 449 aa, Artificial sequence
  An artificially synthesized peptide sequence
QVQLQESGPGLVKPSETLSLTCAVSGHSISHDHAWSWVRQPPGEGLEWIGFISYSGITNYNPSLQGRVTISRDNSKNTLYLQMNSLRAEDTAVYYCARSLARTTAMDYWGEGTLVTVSSAKTTAPSVYPLAPVCGDTTGSSVTLGCLVKGYFPEPVTLTWNSGSLSSGVHTFPAVLQSDLYTLSSSVTVTSSTWPSQSITCNVAHPASSTKVDKKIEPRGPTIKPCPPCKCPAPNLLGGPDVFIFPPKIKDVLYISLEPIVTCVVVDVSEDDPDVQISWFVNNVEVHTAQTQTHREDYNSTLRVVSALPIQHQDWMSGKEFKCKVNNDDYPAPIERTISKPKGSVRAPQVYVLPPPEEEMTKKQVTLTCMVTDFMPEDIYVEWTNNGKTELNYKNTEPVLDSDGSYFMYSKLRVEKKNWVERNSYSCSVVHEGLKFHHTTKSFSRTPGK

SEQ ID NO: 131 - DNA, 34 bp, Artificial sequence
  An artificially synthesized peptide sequence
ataacttcgtatagcatacattatacgaagttat

SEQ ID NO: 132 - DNA, 21 bp, Artificial sequence
  An artificially synthesized peptide sequence
acagggccttagactcacagc

SEQ ID NO: 133 - DNA, 22 bp, Artificial sequence
  An artificially synthesized peptide sequence
aacttgctcccgacactactgg

SEQ ID NO: 134 - DNA, 22 bp, Artificial sequence
  An artificially synthesized peptide sequence
tctgcagtagccttcaaagagc

SEQ ID NO: 135 - DNA, 21 bp, Artificial sequence
  An artificially synthesized peptide sequence
aaccagacagtgtcacattcc

SEQ ID NO: 136 - DNA, 22 bp, Artificial sequence
  An artificially synthesized peptide sequence
cccggctgcggagccgctctgc

SEQ ID NO: 137 - DNA, 21 bp, Artificial sequence
  An artificially synthesized peptide sequence
acagtgatgctggaggtcctt

SEQ ID NO: 138 - DNA, 22 bp, Artificial sequence
  An artificially synthesized peptide sequence
agcaacaccgtgaactcctttg